European Patent Application EP 4 624 489 A1, published October 1, 2025. Title: METHOD FOR PRODUCING PROTEIN. Applicant: Chugai Seiyaku Kabushiki Kaisha. The sequence listing filed with the application follows.

SEQUENCE LISTING (60 sequences)

SEQ ID NO: 1 - protein, 330 aa, synthetic construct [sequence omitted]

SEQ ID NO: 2 - protein, 326 aa, synthetic construct
  source 1..326: note = an artificially synthesized sequence
ASTKGPSVFPLAPCSRSTSESTAALGCLVKDYFPEPVTVSWNSGALTSGVHTFPAVLQSSGLYSLSSVVTVPSSNFGTQTYTCNVDHKPSNTKVDKTVERKCCVECPPCPAPPVAGPSVFLFPPKPKDTLMISRTPEVTCVVVDVSHEDPEVQFNWYVDGVEVHNAKTKPREEQFNSTFRVVSVLTVVHQDWLNGKEYKCKVSNKGLPAPIEKTISKTKGQPREPQVYTLPPSREEMTKNQVSLTCLVKGFYPSDIAVEWESNGQPENNYKTTPPMLDSDGSFFLYSKLTVDKSRWQQGNVFSCSVMHEALHNHYTQKSLSLSPGK

SEQ ID NO: 3 - protein, 377 aa, synthetic construct
  source 1..377: note = an artificially synthesized sequence
ASTKGPSVFPLAPCSRSTSGGTAALGCLVKDYFPEPVTVSWNSGALTSGVHTFPAVLQSSGLYSLSSVVTVPSSSLGTQTYTCNVNHKPSNTKVDKRVELKTPLGDTTHTCPRCPEPKSCDTPPPCPRCPEPKSCDTPPPCPRCPEPKSCDTPPPCPRCPAPELLGGPSVFLFPPKPKDTLMISRTPEVTCVVVDVSHEDPEVQFKWYVDGVEVHNAKTKPREEQYNSTFRVVSVLTVLHQDWLNGKEYKCKVSNKALPAPIEKTISKTKGQPREPQVYTLPPSREEMTKNQVSLTCLVKGFYPSDIAVEWESSGQPENNYNTTPPMLDSDGSFFLYSKLTVDKSRWQQGNIFSCSVMHEALHNRFTQKSLSLSPGK

SEQ ID NO: 4 - protein, 327 aa, synthetic construct
  source 1..327: note = an artificially synthesized sequence
ASTKGPSVFPLAPCSRSTSESTAALGCLVKDYFPEPVTVSWNSGALTSGVHTFPAVLQSSGLYSLSSVVTVPSSSLGTKTYTCNVDHKPSNTKVDKRVESKYGPPCPSCPAPEFLGGPSVFLFPPKPKDTLMISRTPEVTCVVVDVSQEDPEVQFNWYVDGVEVHNAKTKPREEQFNSTYRVVSVLTVLHQDWLNGKEYKCKVSNKGLPSSIEKTISKAKGQPREPQVYTLPPSQEEMTKNQVSLTCLVKGFYPSDIAVEWESNGQPENNYKTTPPVLDSDGSFFLYSRLTVDKSRWQEGNVFSCSVMHEALHNHYTQKSLSLSLGK

SEQ ID NO: 5 - protein, 4 aa, synthetic construct
  source 1..4: note = an artificially synthesized sequence
GGGS

SEQ ID NO: 6 - protein, 4 aa, synthetic construct
  source 1..4: note = an artificially synthesized sequence
SGGG

SEQ ID NO: 7 - protein, 5 aa, synthetic construct
  source 1..5: note = an artificially synthesized sequence
GGGGS

SEQ ID NO: 8 - protein, 5 aa, synthetic construct
  source 1..5: note = an artificially synthesized sequence
SGGGG

SEQ ID NO: 9 - protein, 6 aa, synthetic construct
  source 1..6: note = an artificially synthesized sequence
GGGGGS

SEQ ID NO: 10 - protein, 6 aa, synthetic construct
  source 1..6: note = an artificially synthesized sequence
SGGGGG

SEQ ID NO: 11 - protein, 7 aa, synthetic construct
  source 1..7: note = an artificially synthesized sequence
GGGGGGS

SEQ ID NO: 12 - protein, 7 aa, synthetic construct
  source 1..7: note = an artificially synthesized sequence
SGGGGGG

SEQ ID NO: 13 - protein, 207 aa, synthetic construct
  source 1..207: note = an artificially synthesized sequence
MQSGTHWRVLGLCLLSVGVWGQDGNEEMGGITQTPYKVSISGTTVILTCPQYPGSEILWQHNDKNIGGDEDDKNIGSDEDHLSLKEFSELEQSGYYVCYPRGSKPEDANFYLYLRARVCENCMEMDVMSVATIVIVDICITGGLLLLVYYWSKNRKAKAKPVTRGAGAGGRQRGQNKERPPPVPNPDYEPIRKGQRDLYSGLNQRRI

SEQ ID NO: 14 - protein, 72 aa, synthetic construct
  source 1..72: note = an artificially synthesized sequence
SPCPPNSFSSAGGQRTCDICRQCKGVFRTRKECSSTSNAECDCTPGFHCLGAGCSMCEQDCKQGQELTKKGC

SEQ ID NO: 15 - protein, 31 aa, synthetic construct
  source 1..31: note = an artificially synthesized sequence
DCTPGFHCLGAGCSMCEQDCKQGQELTKKGC

SEQ ID NO: 16 - protein, 63 aa, synthetic construct
  source 1..63: note = an artificially synthesized sequence
LQDPCSNCPAGTFCDNNRNQICSPCPPNSFSSAGGQRTCDICRQCKGVFRTRKECSSTSNAEC

SEQ ID NO: 17 - protein, 22 aa, synthetic construct
  source 1..22: note = an artificially synthesized sequence
LQDPCSNCPAGTFCDNNRNQIC

SEQ ID NO: 18 - protein, 11 aa, synthetic construct
  source 1..11: note = an artificially synthesized sequence
VEPKSCGGGGS

SEQ ID NO: 19 - protein, 16 aa, synthetic construct
  source 1..16: note = an artificially synthesized sequence
VEPKSCGGGGSGGGGS

SEQ ID NO: 20 - protein, 6 aa, synthetic construct
  source 1..6: note = an artificially synthesized sequence
VEPKSC

SEQ ID NO: 21 - protein, 88 aa, synthetic construct
  source 1..88: note = an artificially synthesized sequence
MVLASSTTSIHTMLLLLLMLAQPAMARADPCAARPCAHGGRCYAHFSGLVCACAPGYMGARCEFPVHPDGASALPAAPPGLRPGDPQR

SEQ ID NO: 22 - protein, 618 aa, synthetic construct
  source 1..618: note = an artificially synthesized sequence
MVSPRMSGLLSQTVILALIFLPQTRPAGVFELQIHSFGPGPGPGAPRSPCSARLPCRLFFRVCLKPGLSEEAAESPCALGAALSARGPVYTEQPGAPAPDLPLPDGLLQVPFRDAWPGTFSFIIETWREELGDQIGGPAWSLLARVAGRRRLAAGGPWARDIQRAGAWELRFSYRARCEPPAVGTACTRLCRPRSAPSRCGPGLRPCAPLEDECEAPLVCRAGCSPEHGFCEQPGECRCLEGWTGPLCTVPVSTSSCLSPRGPSSATTGCLVPGPGPCDGNPCANGGSCSETPRSFECTCPRGFYGLRCEVSGVTCADGPCFNGGLCVGGADPDSAYICHCPPGFQGSNCEKRVDRCSLQPCRNGGLCLDLGHALRCRCRAGFAGPRCEHDLDDCAGRACANGGTCVEGGGAHRCSCALGFGGRDCRERADPCAARPCAHGGRCYAHFSGLVCACAPGYMGARCEFPVHPDGASALPAAPPGLRPGDPQRYLLPPALGLLVAAGVAGAALLLVHVRRRGHSQDAGSRLLAGTPEPSVHALPDALNNLRTQEGSGDGPSSSVDWNRPEDVDPQGIYVISAPSIYAREVATPLFPPLHTGRAGQRQHLLFPYPSSILSVK

SEQ ID NO: 23 - protein, 220 aa, synthetic construct
  source 1..220: note = an artificially synthesized sequence
CPPCPAPEAAGGPSVFLFPPKPKDTLMISRTPEVTCVVVDVSHEDPEVKFNWYVDGVEVHNAKTKPREEQYASTYRVVSVLTVLHQDWLNGKEYKCKVSNKALPAPIEKTISKAKGQPREPQVYTLPPCRDELTKNQVSLWCLVKGFYPSDIAVEWESNGQPENNYKTTPPVLDSDGSFFLYSKLTVDKSRWQQGNVFSCSVLHEALHAHYTRKELSLSP

SEQ ID NO: 24 - protein, 220 aa, synthetic construct
  source 1..220: note = an artificially synthesized sequence
CPPCPAPEAAGGPSVFLFPPKPKDTLMISRTPEVTCVVVDVSHEDPEVKFNWYVDGVEVHNAKTKPREEQYASTYRVVSVLTVLHQDWLNGKEYKCKVSNKALPAPIEKTISKAKGQPREPQVCTLPPSRDELTKNQVSLSCAVKGFYPSDIAVEWESNGQPENNYKTTPPVLDSDGSFFLVSKLTVDKSRWQQGNVFSCSVLHEALHAHYTRKELSLSP

SEQ ID NO: 25 - protein, 220 aa, synthetic construct
  source 1..220: note = an artificially synthesized sequence
CPPCPAPEAAGGPSVFLFPPKPKDTLMISRTPEVTCVVVDVSHEDPEVKFNWYVDGVEVHNAKTKPREEQYASTYRVVSVLTVLHQDWLNGKEYKCKVSNKALPAPIEKTISKAKGQPREPQVYTLPPCRDELTKNQVSLWCLVKGFYPSDIAVEWESNGQPENNYKTTPPVLDSDGSFFLYSKLTVDKSRWQEGNVFSCSVLHEALHAHYTRKELSLSP

SEQ ID NO: 26 - protein, 220 aa, synthetic construct
  source 1..220: note = an artificially synthesized sequence
CPPCPAPEAAGGPSVFLFPPKPKDTLMISRTPEVTCVVVDVSHEDPEVKFNWYVDGVEVHNAKTKPREEQYASTYRVVSVLTVLHQDWLNGKEYKCKVSNKALPAPIEKTISKAKGQPREPQVCTLPPSRDELTKNQVSLSCAVKGFYPSDIAVEWESNGQPENNYKTTPPVLDSDGSFFLVSKLTVDKSRWQEGNVFSCSVLHEALHAHYTRKELSLSP

SEQ ID NO: 27 - protein, 5 aa, synthetic construct
  source 1..5: note = an artificially synthesized sequence
NVWFH

SEQ ID NO: 28 - protein, 19 aa, synthetic construct
  source 1..19: note = an artificially synthesized sequence
QIKDYYNAYAAYYAPSVKG

SEQ ID NO: 29 - protein, 17 aa, synthetic construct
  source 1..17: note = an artificially synthesized sequence
VHYASASTLLPAEGVDA

SEQ ID NO: 30 - protein, 16 aa, synthetic construct
  source 1..16: note = an artificially synthesized sequence
QPSQEVVHMNRNTYLH

SEQ ID NO: 31 - protein, 7 aa, synthetic construct
  source 1..7: note = an artificially synthesized sequence
KVSNRFP

SEQ ID NO: 32 - protein, 9 aa, synthetic construct
  source 1..9: note = an artificially synthesized sequence
AQGTSHPFT

SEQ ID NO: 33 - protein, 5 aa, synthetic construct
  source 1..5: note = an artificially synthesized sequence
NVWFH

SEQ ID NO: 34 - protein, 19 aa, synthetic construct
  source 1..19: note = an artificially synthesized sequence
QIKDYYNAYAGYYHPSVKG

SEQ ID NO: 35 - protein, 17 aa, synthetic construct
  source 1..17: note = an artificially synthesized sequence
VHYAAASQLLPAEGVDA

SEQ ID NO: 36 - protein, 128 aa, synthetic construct
  source 1..128: note = an artificially synthesized sequence
QVQLVESGGGLVQPGRSLRLSCAASGFKFSNVWFHWVRQAPGKGLEWVAQIKDYYNAYAAYYAPSVKGRFTISRDDSKNSIYLQMNSLKTEDTAVYYCHYVHYASASTLLPAEGVDAWGQGTTVTVSS

SEQ ID NO: 37 - protein, 112 aa, synthetic construct
  source 1..112: note = an artificially synthesized sequence
DIVMTQSPLSLPVTPGEPASISCQPSQEVVHMNRNTYLHWYQQKPGQAPRLLIYKVSNRFPGVPDRFSGSGSGTDFTLKISRVEAEDVGVYYCAQGTSHPFTFGQGTKLEIK

SEQ ID NO: 38 - protein, 128 aa, synthetic construct
  source 1..128: note = an artificially synthesized sequence
QVQLVESGGGLVQPGRSLRLSCAASGFKFSNVWFHWVRQAPGKGLEWVAQIKDYYNAYAGYYHPSVKGRFTISRDDSKNSIYLQMNSLKTEDTAVYYCHYVHYAAASQLLPAEGVDAWGQGTTVTVSS

SEQ ID NO: 39 - protein, 681 aa, synthetic construct
  source 1..681: note = an artificially synthesized sequence
DIQLTQSPSFLSASVGDRVTITCQSTESVYGSDWLSWYQQKPGQPPKLLIYQASNLEIGVPSRFSGSGSGTDFTLTINSLEAEDAATYYCQGYYSGYIYAFGGGTKVEIKSSASTKGPSVFPLAPSSRSTSESTAALGCLVKDYFPEPVTVSWNSGALTSGVHTFPAVLQSSGLYSLSSVVTVPSSSLGTKTYTCNVDHKPSNTKVDKRVEPKSCGGGGSGGGGSQVQLVESGGGLVQPGRSLRLSCAASGFKFSNVWFHWVRQAPGKGLEWVAQIKDYYNAYAAYYAPSVKGRFTISRDDSKNSIYLQMNSLKTEDTAVYYCHYVHYASASTLLPAEGVDAWGQGTTVTVSSASTKGPSVFPLAPSSKSTSGGTAALGCLVEDYFPEPVTVSWNSGALTSGVHTFPAVLQSSGLYSLSSVVTVPSCSLGTQTYICNVNHKPSNTKVDEKVEPKSCDKTHTCPPCPAPEAAGGPSVFLFPPKPKDTLMISRTPEVTCVVVDVSHEDPEVKFNWYVDGVEVHNAKTKPREEQYASTYRVVSVLTVLHQDWLNGKEYKCKVSNKALPAPIEKTISKAKGQPREPQVYTLPPCRDELTKNQVSLWCLVKGFYPSDIAVEWESNGQPENNYKTTPPVLDSDGSFFLYSKLTVDKSRWQEGNVFSCSVLHEALHAHYTRKELSLSP

SEQ ID NO: 40 - protein, 226 aa, synthetic construct
  source 1..226: note = an artificially synthesized sequence
QVTLRESGPALVKPTQTLTLTCTFSGFSLSSSYDMGWVRQAPGQGLEWMGTIYTGDYSTDYASWAKGRVTISVDRSKNQFSLKLSSVTAADTAVYYCARHTGYGYFGLWGQGTLVTVSSASVAAPSVFIFPPSDEQLKSGTASVVCLLNNFYPREAKVQWKVDNALQSGNSQESVTEQDSKDSTYSLSSTLTLSKADYEKHKVYACEVTHQGLSSPVTKSFNRGEC

SEQ ID NO: 41 - protein, 456 aa, synthetic construct
  source 1..456: note = an artificially synthesized sequence
QVQLVESGGGLVQPGRSLRLSCAASGFKFSNVWFHWVRQAPGKGLEWVAQIKDYYNAYAAYYAPSVKGRFTISRDDSKNSIYLQMNSLKTEDTAVYYCHYVHYASASTLLPAEGVDAWGQGTTVTVSSASTKGPSVFPLAPSSKSTSGGTAALGCLVEDYFPEPVTVSWNSGALTSGVHTFPAVLQSSGLYSLSSVVTVPSCSLGTQTYICNVNHKPSNTKVDEKVEPKSCDKTHTCPPCPAPEAAGGPSVFLFPPKPKDTLMISRTPEVTCVVVDVSHEDPEVKFNWYVDGVEVHNAKTKPREEQYASTYRVVSVLTVLHQDWLNGKEYKCKVSNKALPAPIEKTISKAKGQPREPQVCTLPPSRDELTKNQVSLSCAVKGFYPSDIAVEWESNGQPENNYKTTPPVLDSDGSFFLVSKLTVDKSRWQEGNVFSCSVLHEALHAHYTRKELSLSP

SEQ ID NO: 42 - protein, 219 aa, synthetic construct
  source 1..219: note = an artificially synthesized sequence
DIVMTQSPLSLPVTPGEPASISCQPSQEVVHMNRNTYLHWYQQKPGQAPRLLIYKVSNRFPGVPDRFSGSGSGTDFTLKISRVEAEDVGVYYCAQGTSHPFTFGQGTKLEIKRTVAAPSVFIFPPSDRKLKSGTASVVCLLNNFYPREAKVQWKVDNALQSGNSQESVTEQDSKDSTYSLSSTLTLSKADYEKHKVYACEVTHQGLSSPVTKSFNRGEC

SEQ ID NO: 43 - protein, 681 aa, synthetic construct
  source 1..681: note = an artificially synthesized sequence
DIQLTQSPSFLSASVGDRVTITCQSTESVYGSDWLSWYQQKPGQPPKLLIYQASNLEIGVPSRFSGSGSGTDFTLTINSLEAEDAATYYCQGYYSGYIYAFGGGTKVEIKSSASTKGPSVFPLAPSSRSTSESTAALGCLVKDYFPEPVTVSWNSGALTSGVHTFPAVLQSSGLYSLSSVVTVPSSSLGTKTYTCNVDHKPSNTKVDKRVEPKSCGGGGSGGGGSQVQLVESGGGLVQPGRSLRLSCAASGFKFSNVWFHWVRQAPGKGLEWVAQIKDYYNAYAAYYAPSVKGRFTISRDDSKNSIYLQMNSLKTEDTAVYYCHYVHYASASTLLPAEGVDAWGQGTTVTVSSASTKGPSVFPLAPSSKSTSGGTAALGCLVEDYFPEPVTVSWNSGALTSGVHTFPAVLQSSGLYSLSSVVTVPSCSLGTQTYICNVNHKPSNTKVDEKVEPKSCDKTHTCPPCPAPEAAGGPSVFLFPPKPKDTLMISRTPEVTCVVVDVSHEDPEVKFNWYVDGVEVHNAKTKPREEQYASTYRVVSVLTVLHQDWLNGKEYKCKVSNKALPAPIEKTISKAKGQPREPQVYTLPPCRDELTKNQVSLWCLVKGFYPSDIAVEWESNGQPENNYKTTPPVLDSDGSFFLYSKLTVDKSRWQQGNVFSCSVLHEALHAHYTRKELSLSP

SEQ ID NO: 44 - protein, 456 aa, synthetic construct
  source 1..456: note = an artificially synthesized sequence
QVQLVESGGGLVQPGRSLRLSCAASGFKFSNVWFHWVRQAPGKGLEWVAQIKDYYNAYAAYYAPSVKGRFTISRDDSKNSIYLQMNSLKTEDTAVYYCHYVHYASASTLLPAEGVDAWGQGTTVTVSSASTKGPSVFPLAPSSKSTSGGTAALGCLVEDYFPEPVTVSWNSGALTSGVHTFPAVLQSSGLYSLSSVVTVPSCSLGTQTYICNVNHKPSNTKVDEKVEPKSCDKTHTCPPCPAPEAAGGPSVFLFPPKPKDTLMISRTPEVTCVVVDVSHEDPEVKFNWYVDGVEVHNAKTKPREEQYASTYRVVSVLTVLHQDWLNGKEYKCKVSNKALPAPIEKTISKAKGQPREPQVCTLPPSRDELTKNQVSLSCAVKGFYPSDIAVEWESNGQPENNYKTTPPVLDSDGSFFLVSKLTVDKSRWQQGNVFSCSVLHEALHAHYTRKELSLSP

SEQ ID NO: 45 - protein, 676 aa, synthetic construct
  source 1..676: note = an artificially synthesized sequence
DIQLTQSPSFLSASVGDRVTITCQSTESVYGSDWLSWYQQKPGQPPKLLIYQASNLEIGVPSRFSGSGSGTDFTLTINSLEAEDAATYYCQGYYSGYIYAFGGGTKVEIKSSASTKGPSVFPLAPSSRSTSESTAALGCLVKDYFPEPVTVSWNSGALTSGVHTFPAVLQSSGLYSLSSVVTVPSSSLGTKTYTCNVDHKPSNTKVDKRVEPKSCGGGGSQVQLVESGGGLVQPGRSLRLSCAASGFKFSNVWFHWVRQAPGKGLEWVAQIKDYYNAYAAYYAPSVKGRFTISRDDSKNSIYLQMNSLKTEDTAVYYCHYVHYASASTLLPAEGVDAWGQGTTVTVSSASTKGPSVFPLAPSSKSTSGGTAALGCLVEDYFPEPVTVSWNSGALTSGVHTFPAVLQSSGLYSLSSVVTVPSCSLGTQTYICNVNHKPSNTKVDEKVEPKSCDKTHTCPPCPAPEAAGGPSVFLFPPKPKDTLMISRTPEVTCVVVDVSHEDPEVKFNWYVDGVEVHNAKTKPREEQYASTYRVVSVLTVLHQDWLNGKEYKCKVSNKALPAPIEKTISKAKGQPREPQVYTLPPCRDELTKNQVSLWCLVKGFYPSDIAVEWESNGQPENNYKTTPPVLDSDGSFFLYSKLTVDKSRWQQGNVFSCSVLHEALHAHYTRKELSLSP

SEQ ID NO: 46 - protein, 6 aa, synthetic construct
  source 1..6: note = an artificially synthesized sequence
SSYDMG

SEQ ID NO: 47 - protein, 17 aa, synthetic construct
  source 1..17: note = an artificially synthesized sequence
TIYTGDYSTDYASWAKG

SEQ ID NO: 48 - protein, 9 aa, synthetic construct
  source 1..9: note = an artificially synthesized sequence
HTGYGYFGL

SEQ ID NO: 49 - protein, 13 aa, synthetic construct
  source 1..13: note = an artificially synthesized sequence
QSTESVYGSDWLS

SEQ ID NO: 50 - protein, 7 aa, synthetic construct
  source 1..7: note = an artificially synthesized sequence
QASNLEI

SEQ ID NO: 51 - protein, 10 aa, synthetic construct
  source 1..10: note = an artificially synthesized sequence
QGYYSGYIYA

SEQ ID NO: 52 - protein, 119 aa, synthetic construct
  source 1..119: note = an artificially synthesized sequence
QVTLRESGPALVKPTQTLTLTCTFSGFSLSSSYDMGWVRQAPGQGLEWMGTIYTGDYSTDYASWAKGRVTISVDRSKNQFSLKLSSVTAADTAVYYCARHTGYGYFGLWGQGTLVTVSS

SEQ ID NO: 53 - protein, 110 aa, synthetic construct
  source 1..110: note = an artificially synthesized sequence
DIQLTQSPSFLSASVGDRVTITCQSTESVYGSDWLSWYQQKPGQPPKLLIYQASNLEIGVPSRFSGSGSGTDFTLTINSLEAEDAATYYCQGYYSGYIYAFGGGTKVEIK

SEQ ID NO: 54 - protein, 698 aa, synthetic construct
  source 1..698: note = Ab2-chain1_split
MDMRVPAQLLGLLLLWLPGARCDIQLTQSPSFLSASVGDRVTITCQSTESVYGSDWLSWYQQKPGQPPKLLIYQASNLEIGVPSRFSGSGSGTDFTLTINSLEAEDAATYYCQGYYSGYIYAFGGGTKVEIKSSASTKGPSVFPLAPSSRSTSESTAALGCLVKDYFPEPVTVSWNSGALTSGVHTFPAVLQSSGLYSLSSVVTVPSSSLGTKTYTCNVDHKPSNTKVDKRVEPKSCGGGGSQVQLVESGGGLVQPGRSLRLSCAASGFKFSNVWFHWVRQAPGKGLEWVAQIKDYYNAYAAYYAPSVKGRFTISRDDSKNSIYLQMNSLKTEDTAVYYCHYVHYASASTLLPAEGVDAWGQGTTVTVSSASTKGPSVFPLAPSSKSTSGGTAALGCLVEDYFPEPVTVSWNSGALTSGVHTFPAVLQSSGLYSLSSVVTVPSCSLGTQTYICNVNHKPSNTKVDEKVEPKSCDKTHTCPPCPAPEAAGGPSVFLFPPKPKDTLMISRTPEVTCVVVDVSHEDPEVKFNWYVDGVEVHNAKTKPREEQYASTYRVVSVLTVLHQDWLNGKEYKCKVSNKALPAPIEKTISKAKGQPREPQVYTLPPCRDELTKNQVSLWCLVKGFYPSDIAVEWESNGQPENNYKTTPPVLDSDGSFFLYSKLTVDKSRWQQGNVFSCSVLHEALHAHYTRKELSLSP

SEQ ID NO: 55 - protein, 245 aa, synthetic construct
  source 1..245: note = chain2
MGWSCIILFLVATATGVHSQVTLRESGPALVKPTQTLTLTCTFSGFSLSSSYDMGWVRQAPGQGLEWMGTIYTGDYSTDYASWAKGRVTISVDRSKNQFSLKLSSVTAADTAVYYCARHTGYGYFGLWGQGTLVTVSSASVAAPSVFIFPPSDEQLKSGTASVVCLLNNFYPREAKVQWKVDNALQSGNSQESVTEQDSKDSTYSLSSTLTLSKADYEKHKVYACEVTHQGLSSPVTKSFNRGEC

SEQ ID NO: 56 - protein, 475 aa, synthetic construct
  source 1..475: note = chain3
MGWSCIILFLVATATGVHSQVQLVESGGGLVQPGRSLRLSCAASGFKFSNVWFHWVRQAPGKGLEWVAQIKDYYNAYAAYYAPSVKGRFTISRDDSKNSIYLQMNSLKTEDTAVYYCHYVHYASASTLLPAEGVDAWGQGTTVTVSSASTKGPSVFPLAPSSKSTSGGTAALGCLVEDYFPEPVTVSWNSGALTSGVHTFPAVLQSSGLYSLSSVVTVPSCSLGTQTYICNVNHKPSNTKVDEKVEPKSCDKTHTCPPCPAPEAAGGPSVFLFPPKPKDTLMISRTPEVTCVVVDVSHEDPEVKFNWYVDGVEVHNAKTKPREEQYASTYRVVSVLTVLHQDWLNGKEYKCKVSNKALPAPIEKTISKAKGQPREPQVCTLPPSRDELTKNQVSLSCAVKGFYPSDIAVEWESNGQPENNYKTTPPVLDSDGSFFLVSKLTVDKSRWQQGNVFSCSVMHEALHNHYTQKSLSLSP

SEQ ID NO: 57 - protein, 238 aa, synthetic construct
  source 1..238: note = chain4
MGWSCIILFLVATATGVHSDIVMTQSPLSLPVTPGEPASISCQPSQEVVHMNRNTYLHWYQQKPGQAPRLLIYKVSNRFPGVPDRFSGSGSGTDFTLKISRVEAEDVGVYYCAQGTSHPFTFGQGTKLEIKRTVAAPSVFIFPPSDRKLKSGTASVVCLLNNFYPREAKVQWKVDNALQSGNSQESVTEQDSKDSTYSLSSTLTLSKADYEKHKVYACEVTHQGLSSPVTKSFNRGEC

SEQ ID NO: 58 - protein, 216 aa, synthetic construct
  source 1..216: note = Ab2-chain1_split_Fc
PAPEAAGGPSVFLFPPKPKDTLMISRTPEVTCVVVDVSHEDPEVKFNWYVDGVEVHNAKTKPREEQYASTYRVVSVLTVLHQDWLNGKEYKCKVSNKALPAPIEKTISKAKGQPREPQVYTLPPCRDELTKNQVSLWCLVKGFYPSDIAVEWESNGQPENNYKTTPPVLDSDGSFFLYSKLTVDKSRWQQGNVFSCSVLHEALHAHYTRKELSLSP

SEQ ID NO: 59 - protein, 216 aa, synthetic construct
  source 1..216: note = chain3_Fc
PAPEAAGGPSVFLFPPKPKDTLMISRTPEVTCVVVDVSHEDPEVKFNWYVDGVEVHNAKTKPREEQYASTYRVVSVLTVLHQDWLNGKEYKCKVSNKALPAPIEKTISKAKGQPREPQVCTLPPSRDELTKNQVSLSCAVKGFYPSDIAVEWESNGQPENNYKTTPPVLDSDGSFFLVSKLTVDKSRWQQGNVFSCSVMHEALHNHYTQKSLSLSP

SEQ ID NO: 60 - protein, 475 aa, synthetic construct
  source 1..475: note = chain3
MGWSCIILFLVATATGVHSQVQLVESGGGLVQPGRSLRLSCAASGFKFSNVWFHWVRQAPGKGLEWVAQIKDYYNAYAAYYAPSVKGRFTISRDDSKNSIYLQMNSLKTEDTAVYYCHYVHYASASTLLPAEGVDAWGQGTTVTVSSASTKGPSVFPLAPSSKSTSGGTAALGCLVEDYFPEPVTVSWNSGALTSGVHTFPAVLQSSGLYSLSSVVTVPSCSLGTQTYICNVNHKPSNTKVDEKVEPKSCDKTHTCPPCPAPEAAGGPSVFLFPPKPKDTLMISRTPEVTCVVVDVSHEDPEVKFNWYVDGVEVHNAKTKPREEQYASTYRVVSVLTVLHQDWLNGKEYKCKVSNKALPAPIEKTISKAKGQPREPQVCTLPPSRDELTKNQVSLSCAVKGFYPSDIAVEWESNGQPENNYKTTPPVLDSDGSFFLVSKLTVDKSRWQQGNVFSCSVLHEALHAHYTRKELSLSP